European Patent Application EP 4 379 376 A2, published June 5, 2024. Title: COMPOSITIONS AND METHODS FOR TREATMENT OF HEREDITARY CYSTATIN C AMYLOID ANGIOPATHY ( HCCAA) AND OTHER NEURODEGENERATIVE DISORDERS ASSOCIATED WITH ABERRANT AMYLOID DEPOSITS. Applicant: The Children's Hospital of Philadelphia. Application EP 24155226.4, filed September 7, 2018. The sequence listing filed with the application follows.

SEQUENCE LISTING (4 sequences)

SEQ ID NO: 1 - DNA, 35 bp, synthetic construct
  misc_feature 1..35: note = primer
  source 1..35: mol_type = other DNA
gatcgaattcgccaccatggccgggcccctgcgcg

SEQ ID NO: 2 - DNA, 66 bp, synthetic construct
  misc_feature 1..66: note = primer
  source 1..66: mol_type = other DNA
tcgcggccgcctacagatcctcttctgagatgagtttttgttcggcgtcctgacaggtggatttcg

SEQ ID NO: 3 - DNA, 45 bp, synthetic construct
  misc_feature 1..45: note = primer
  source 1..45: mol_type = other DNA
gtgaactacttcttggacgtcgagcagggccgaaccacgtgtacc

SEQ ID NO: 4 - DNA, 45 bp, synthetic construct
  misc_feature 1..45: note = primer
  source 1..45: mol_type = other DNA
ggtacacgtggttcggccctgctcgacgtccaagaagtagttcac